European Patent Specification EP 3 769 781 B1, published April 19, 2023. Title: STABLE ANTI-IFNAR1 FORMULATION. Applicant: DEPAZ, ROBERTO DEJESUS, NATALIE BEE, JARED. Application 62/207,164. The sequence listing filed with the application follows.

SEQUENCE LISTING (2 sequences)

SEQ ID NO: 1 - protein, 117 aa, Artificial Sequence
  Description of Artificial Sequence: Synthetic polypeptide
EVQLVQSGAEVKKPGESLKISCKGSGYIFTNYWIAWVRQMPGKCLESMGIIYPGDSDIRYSPSFQGQVTISADKSITTAYLQWSSLKASDTAMYYCARHDIEGFDYWGRGTLVTVSS

SEQ ID NO: 2 - protein, 108 aa, Artificial Sequence [sequence omitted]